European Patent Application EP 4 155 396 A1, published March 29, 2023. Title: PHYTASE MUTANT. Applicant: QINGDAO VLAND BIOTECH GROUP CO., LTD. Application EP21809654.3. The sequence listing filed with the application follows.

SEQUENCE LISTING (28 sequences)

SEQ ID NO: 1 - protein, 410 aa, Escherichia coli
QSEPELKLESVVIVSRHGVRAPTKATQLMQDVTPDAWPTWPVKLGWLTPRGGELIAYLGHYQRQRLVADGLLAKKGCPQSGQVAIIADVDERTRKTGEAFAAGLAPDCAITVHTQADTSSPDPLFNPLKTGVCQLDNANVTDAILSRAGGSIADFTGHRQTAFRELERVLNFPQSNLCLKREKQDESCSLTQALPSELKVSADNVSLTGAVSLASMLTEIFLLQQAQGMPEPGWGRITDSHQWNTLLSLHNAQFYLLQRTPEVARSRATPLLDLIKTALTPHPPQKQAYGVTLPTSVLFIAGHDTNLANLGGALELNWTLPGQPDNTPPGGELVFERWRRLSDNSQWIQVSLVFQTLQQMRDKTPLSLNTPPGEVKLTLAGCEERNAQGMCSLAGFTQIVNEARIPACSL

SEQ ID NO: 2 - DNA, 1233 bp, Escherichia coli
cagagtgagccggagctgaagctggaaagtgtggtgattgtcagtcgtcatggtgtgcgtgctccaaccaaggccacgcaactgatgcaggatgtcaccccagacgcatggccaacctggccggtaaaactgggttggctgacaccgcgcggtggtgagctaatcgcctatctcggacattaccaacgccagcgtctggtagccgacggattgctggcgaaaaagggctgcccgcagtctggtcaggtcgcgattattgctgatgtcgacgagcgtacccgtaaaacaggcgaagccttcgccgccgggctggcacctgactgtgcaataaccgtacatacccaggcagatacgtccagtcccgatccgttatttaatcctctaaaaactggcgtttgccaactggataacgcgaacgtgactgacgcgatcctcagcagggcaggagggtcaattgctgactttaccgggcatcggcaaacggcgtttcgcgaactggaacgggtgcttaattttccgcaatcaaacttgtgccttaaacgtgagaaacaggacgaaagctgttcattaacgcaggcattaccatcggaactcaaggtgagcgccgacaatgtctcattaaccggtgcggtaagcctcgcatcaatgctgacggagatatttctcctgcaacaagcacagggaatgccggagccggggtggggaaggatcaccgattcacaccagtggaacaccttgctaagtttgcataacgcgcaattttatttgctacaacgcacgccagaggttgcccgcagccgcgccaccccgttattagatttgatcaagacagcgttgacgccccatccaccgcaaaaacaggcgtatggtgtgacattacccacttcagtgctgtttatcgccggacacgatactaatctggcaaatctcggcggcgcactggagctcaactggacgcttcccggtcagccggataacacgccgccaggtggtgaactggtgtttgaacgctggcgtcggctaagcgataacagccagtggattcaggtttcgctggtcttccagactttacagcagatgcgtgataaaacgccgctgtcattaaatacgccgcccggagaggtgaaactgaccctggcaggatgtgaagagcgaaatgcgcagggcatgtgttcgttggcaggttttacgcaaatcgtgaatgaagcacgcataccggcgtgcagtttgtaa

SEQ ID NO: 3 - protein, 410 aa, Artificial Sequence
  Phytase mutant
QSEPELKLESVVIVSRHGVRAPTKATQLMQDVTPDAWPTWPVKLGELTPRGGELIAYLGHYWRQRLVADELLPKKGCPQSGQVAIIADVDERTRKTGEAFAAGLAPDCAITVHHQADTSSPDPLFNPLKTGVCQLDVANVTRAILERAGGSIADFTGHYQTAFRELERVLNFPQSNLCLKREKQDESCSLTQALPSELKVSADNVSLTGAVSLASMLTEIFLLQQAQGMPEPGWGRITDSHQWNTLLSLHNAQFDLLQRTPEVARSRATPLLDLIKTALTPHPPQKQAYGVTLPTSVLFIAGHDTNLANLGGALELNWTLPGQPDNTPPGGELVFERWRRLSDNSQWIQVSLVFQTLQQMRDKTPLSLNTPPGEVKLTLAGCEERNAQGMCSLAGFTQIVNEARIPACSL

SEQ ID NO: 4 - DNA, 1230 bp, Artificial Sequence
  Nucleotide sequence encoding phytase mutant
caatctgaaccagaattgaagttggaatctgttgttattgtttcccgtcacggtgttagagccccaactaaggctactcaattgatgcaagatgttactccagatgcttggccaacttggccagttaagttgggtgaattgactccaagaggtggtgaattgattgcttacttgggtcattactggagacaaagattggttgctgatgaattgttgccaaagaagggttgtccacaatctggtcaagttgctattattgctgatgttgatgaacgcactagaaagaccggtgaggcttttgctgctggtttggctccagattgtgctattactgttcatcatcaagctgatacttcttccccagatccattgtttaacccattgaagactggtgtttgtcaattggatgttgctaacgttactagagctattttggaaagagctggtggttctattgctgattttactggtcattaccaaaccgcctttcgtgaattggaaagagttttgaactttccacaatccaacttgtgtttgaagagagaaaagcaagatgagtcctgttccttgacccaagctcttccatctgaattgaaggtttctgctgataacgtttctttgactggtgctgtttctttggcttctatgttgactgaaattttcttgttgcagcaggctcaaggtatgccagaaccaggttggggtagaattactgattctcatcaatggaacactttgttgtctttgcataacgctcaatttgacttgttgcaaagaactccagaagttgctagatctagagctactccattgttggatttgattaagactgctttgactccacatccaccacaaaagcaggcttacggtgttactttgccaacttctgttttgtttattgccggtcatgataccaacttggctaacttgggtggtgctttggaattgaactggactttgccaggtcaaccagataacactccaccaggtggtgaattggtttttgaaagatggagaagattgtccgataactctcaatggattcaagtttctttggtctttcagaccttgcagcaaatgagagataagactccattgtctttgaacactccaccaggtgaagttaagttgactttggctggttgtgaagaaagaaacgctcaaggtatgtgttctttggctggttttactcaaattgtcaacgaggctagaatcccagcttgttctttg

SEQ ID NO: 5 - protein, 410 aa, Artificial Sequence
  Phytase mutant
QSEPELKLESVVIVSRHGVRAPTKATQLMQDVTPDPWPTWPVKLGELTPRGGELIAYLGHYWRQRLVADELLPKKGCPQSGQVAIIADVDERTRKTGEAFAAGLAPDCAITVHHQADTSSPDPLFNPLKTGVCQLDVANVTRAILERAGGSIADFTGHYQTAFRELERVLNFPQSNLCLKREKQDESCSLTQALPSELKVSADNVSLTGAVSLASMLTEIFLLQQAQGMPEPGWGRITDSHQWNTLLSLHNAQFDLLQRTPEVARSRATPLLDLIKTALTPHPPQKQAYGVTLPTSVLFIAGHDTNLANLGGALELNWTLPGQPDNTPPGGELVFERWRRLSDNSQWIQVSLVFQTLQQMRDKTPLSLNTPPGEVKLTLAGCEERNAQGMCSLAGFTQIVNEARIPACSL

SEQ ID NO: 6 - DNA, 1230 bp, Artificial Sequence
  Nucleotide sequence encoding phytase mutant
caatctgaaccagaattgaagttggaatctgttgttattgtttcccgtcacggtgttagagccccaactaaggctactcaattgatgcaagatgttactccagatccatggccaacttggccagttaagttgggtgaattgactccaagaggtggtgaattgattgcttacttgggtcattactggagacaaagattggttgctgatgaattgttgccaaagaagggttgtccacaatctggtcaagttgctattattgctgatgttgatgaacgcactagaaagaccggtgaggcttttgctgctggtttggctccagattgtgctattactgttcatcatcaagctgatacttcttccccagatccattgtttaacccattgaagactggtgtttgtcaattggatgttgctaacgttactagagctattttggaaagagctggtggttctattgctgattttactggtcattaccaaaccgcctttcgtgaattggaaagagttttgaactttccacaatccaacttgtgtttgaagagagaaaagcaagatgagtcctgttccttgacccaagctcttccatctgaattgaaggtttctgctgataacgtttctttgactggtgctgtttctttggcttctatgttgactgaaattttcttgttgcagcaggctcaaggtatgccagaaccaggttggggtagaattactgattctcatcaatggaacactttgttgtctttgcataacgctcaatttgacttgttgcaaagaactccagaagttgctagatctagagctactccattgttggatttgattaagactgctttgactccacatccaccacaaaagcaggcttacggtgttactttgccaacttctgttttgtttattgccggtcatgataccaacttggctaacttgggtggtgctttggaattgaactggactttgccaggtcaaccagataacactccaccaggtggtgaattggtttttgaaagatggagaagattgtccgataactctcaatggattcaagtttctttggtctttcagaccttgcagcaaatgagagataagactccattgtctttgaacactccaccaggtgaagttaagttgactttggctggttgtgaagaaagaaacgctcaaggtatgtgttctttggctggttttactcaaattgtcaacgaggctagaatcccagcttgttctttg

SEQ ID NO: 7 - protein, 410 aa, Artificial Sequence
  Phytase mutant
QSEPELKLESVVIVSRHGVRAPTKATQLMQDVTPDAWPTWPVKLGELTPRGGELIAYLGHYWRQRLVADELLPKKGCPQSGQVAIIADVDERTRKTGEAFAAGLAPDCAITVHHQADTSSPDPLFEPLKTGVCQLDVANVTRAILERAGGSIADFTGHYQTAFRELERVLNFPQSNLCLKREKQDESCSLTQALPSELKVSADNVSLTGAVSLASMLTEIFLLQQAQGMPEPGWGRITDSHQWNTLLSLHNAQFDLLQRTPEVARSRATPLLDLIKTALTPHPPQKQAYGVTLPTSVLFIAGHDTNLANLGGALELNWTLPGQPDNTPPGGELVFERWRRLSDNSQWIQVSLVFQTLQQMRDKTPLSLNTPPGEVKLTLAGCEERNAQGMCSLAGFTQIVNEARIPACSL

SEQ ID NO: 8 - DNA, 1230 bp, Artificial Sequence
  Nucleotide sequence encoding phytase mutant
caatctgaaccagaattgaagttggaatctgttgttattgtttcccgtcacggtgttagagccccaactaaggctactcaattgatgcaagatgttactccagatgcttggccaacttggccagttaagttgggtgaattgactccaagaggtggtgaattgattgcttacttgggtcattactggagacaaagattggttgctgatgaattgttgccaaagaagggttgtccacaatctggtcaagttgctattattgctgatgttgatgaacgcactagaaagaccggtgaggcttttgctgctggtttggctccagattgtgctattactgttcatcatcaagctgatacttcttccccagatccattgtttgagccattgaagactggtgtttgtcaattggatgttgctaacgttactagagctattttggaaagagctggtggttctattgctgattttactggtcattaccaaaccgcctttcgtgaattggaaagagttttgaactttccacaatccaacttgtgtttgaagagagaaaagcaagatgagtcctgttccttgacccaagctcttccatctgaattgaaggtttctgctgataacgtttctttgactggtgctgtttctttggcttctatgttgactgaaattttcttgttgcagcaggctcaaggtatgccagaaccaggttggggtagaattactgattctcatcaatggaacactttgttgtctttgcataacgctcaatttgacttgttgcaaagaactccagaagttgctagatctagagctactccattgttggatttgattaagactgctttgactccacatccaccacaaaagcaggcttacggtgttactttgccaacttctgttttgtttattgccggtcatgataccaacttggctaacttgggtggtgctttggaattgaactggactttgccaggtcaaccagataacactccaccaggtggtgaattggtttttgaaagatggagaagattgtccgataactctcaatggattcaagtttctttggtctttcagaccttgcagcaaatgagagataagactccattgtctttgaacactccaccaggtgaagttaagttgactttggctggttgtgaagaaagaaacgctcaaggtatgtgttctttggctggttttactcaaattgtcaacgaggctagaatcccagcttgttctttg

SEQ ID NO: 9 - protein, 410 aa, Artificial Sequence
  Phytase mutant
QSEPELKLESVVIVSRHGVRAPTKATQLMQDVTPDAWPTWPVKLGELTPRGGELIAYLGHYWRQRLVADELLPKKGCPQSGQVAIIADVDERTRKTGEAFAAGLAPDCAITVHHQADTSSPDPLFNPLKTGVCQLDVANVTRAILERAGGSIADFTGHYQTAFRELERVLNFPQSNLCLKREKQDESCSLTQALPSELKVSADNVSLTGAWSLASMLTEIFLLQQAQGMPEPGWGRITDSHQWNTLLSLHNAQFDLLQRTPEVARSRATPLLDLIKTALTPHPPQKQAYGVTLPTSVLFIAGHDTNLANLGGALELNWTLPGQPDNTPPGGELVFERWRRLSDNSQWIQVSLVFQTLQQMRDKTPLSLNTPPGEVKLTLAGCEERNAQGMCSLAGFTQIVNEARIPACSL

SEQ ID NO: 10 - DNA, 1230 bp, Artificial Sequence
  Nucleotide sequence encoding phytase mutant
caatctgaaccagaattgaagttggaatctgttgttattgtttcccgtcacggtgttagagccccaactaaggctactcaattgatgcaagatgttactccagatgcttggccaacttggccagttaagttgggtgaattgactccaagaggtggtgaattgattgcttacttgggtcattactggagacaaagattggttgctgatgaattgttgccaaagaagggttgtccacaatctggtcaagttgctattattgctgatgttgatgaacgcactagaaagaccggtgaggcttttgctgctggtttggctccagattgtgctattactgttcatcatcaagctgatacttcttccccagatccattgtttaacccattgaagactggtgtttgtcaattggatgttgctaacgttactagagctattttggaaagagctggtggttctattgctgattttactggtcattaccaaaccgcctttcgtgaattggaaagagttttgaactttccacaatccaacttgtgtttgaagagagaaaagcaagatgagtcctgttccttgacccaagctcttccatctgaattgaaggtttctgctgataacgtttctttgactggtgcttggtctttggcttctatgttgactgaaattttcttgttgcagcaggctcaaggtatgccagaaccaggttggggtagaattactgattctcatcaatggaacactttgttgtctttgcataacgctcaatttgacttgttgcaaagaactccagaagttgctagatctagagctactccattgttggatttgattaagactgctttgactccacatccaccacaaaagcaggcttacggtgttactttgccaacttctgttttgtttattgccggtcatgataccaacttggctaacttgggtggtgctttggaattgaactggactttgccaggtcaaccagataacactccaccaggtggtgaattggtttttgaaagatggagaagattgtccgataactctcaatggattcaagtttctttggtctttcagaccttgcagcaaatgagagataagactccattgtctttgaacactccaccaggtgaagttaagttgactttggctggttgtgaagaaagaaacgctcaaggtatgtgttctttggctggttttactcaaattgtcaacgaggctagaatcccagcttgttctttg

SEQ ID NO: 11 - protein, 410 aa, Artificial Sequence
  Phytase mutant
QSEPELKLESVVIVSRHGVRAPTKATQLMQDVTPDAWPTWPVKLGELTPRGGELIAYLGHYWRQRLVADELLPKKGCPQSGQVAIIADVDERTRKTGEAFAAGLAPDCAITVHHQADTSSPDPLFNPLKTGVCQLDVANVTRAILERAGGSIADFTGHYQTAFRELERVLNFPQSNLCLKREKQDESCSLTQALPSELKVSADNVSLTGAVSLASMLTEIFLLQQAQGMPEPGWGRITDSHQWNTLLSLHNAYFDLLQRTPEVARSRATPLLDLIKTALTPHPPQKQAYGVTLPTSVLFIAGHDTNLANLGGALELNWTLPGQPDNTPPGGELVFERWRRLSDNSQWIQVSLVFQTLQQMRDKTPLSLNTPPGEVKLTLAGCEERNAQGMCSLAGFTQIVNEARIPACSL

SEQ ID NO: 12 - DNA, 1230 bp, Artificial Sequence
  Nucleotide sequence encoding phytase mutant
caatctgaaccagaattgaagttggaatctgttgttattgtttcccgtcacggtgttagagccccaactaaggctactcaattgatgcaagatgttactccagatgcttggccaacttggccagttaagttgggtgaattgactccaagaggtggtgaattgattgcttacttgggtcattactggagacaaagattggttgctgatgaattgttgccaaagaagggttgtccacaatctggtcaagttgctattattgctgatgttgatgaacgcactagaaagaccggtgaggcttttgctgctggtttggctccagattgtgctattactgttcatcatcaagctgatacttcttccccagatccattgtttaacccattgaagactggtgtttgtcaattggatgttgctaacgttactagagctattttggaaagagctggtggttctattgctgattttactggtcattaccaaaccgcctttcgtgaattggaaagagttttgaactttccacaatccaacttgtgtttgaagagagaaaagcaagatgagtcctgttccttgacccaagctcttccatctgaattgaaggtttctgctgataacgtttctttgactggtgctgtttctttggcttctatgttgactgaaattttcttgttgcagcaggctcaaggtatgccagaaccaggttggggtagaattactgattctcatcaatggaacactttgttgtctttgcataacgcttactttgacttgttgcaaagaactccagaagttgctagatctagagctactccattgttggatttgattaagactgctttgactccacatccaccacaaaagcaggcttacggtgttactttgccaacttctgttttgtttattgccggtcatgataccaacttggctaacttgggtggtgctttggaattgaactggactttgccaggtcaaccagataacactccaccaggtggtgaattggtttttgaaagatggagaagattgtccgataactctcaatggattcaagtttctttggtctttcagaccttgcagcaaatgagagataagactccattgtctttgaacactccaccaggtgaagttaagttgactttggctggttgtgaagaaagaaacgctcaaggtatgtgttctttggctggttttactcaaattgtcaacgaggctagaatcccagcttgttctttg

SEQ ID NO: 13 - protein, 410 aa, Artificial Sequence
  Phytase mutant
QSEPELKLESVVIVSRHGVRAPTKATQLMQDVTPDAWPTWPVKLGELTPRGGELIAYLGHYWRQRLVADELLPKKGCPQSGQVAIIADVDERTRKTGEAFAAGLAPDCAITVHHQADTSSPDPLFNPLKTGVCQLDVANVTRAILERAGGSIADFTGHYQTAFRELERVLNFPQSNLCLKREKQDESCSLTQALPSELKVSADNVSLTGAVSLASMLTEIFLLQQAQGMPEPGWGRITDSHQWNTLLSLHNAQFDLLERTPEVARSRATPLLDLIKTALTPHPPQKQAYGVTLPTSVLFIAGHDTNLANLGGALELNWTLPGQPDNTPPGGELVFERWRRLSDNSQWIQVSLVFQTLQQMRDKTPLSLNTPPGEVKLTLAGCEERNAQGMCSLAGFTQIVNEARIPACSL

SEQ ID NO: 14 - DNA, 1230 bp, Artificial Sequence
  Nucleotide sequence encoding phytase mutant
caatctgaaccagaattgaagttggaatctgttgttattgtttcccgtcacggtgttagagccccaactaaggctactcaattgatgcaagatgttactccagatgcttggccaacttggccagttaagttgggtgaattgactccaagaggtggtgaattgattgcttacttgggtcattactggagacaaagattggttgctgatgaattgttgccaaagaagggttgtccacaatctggtcaagttgctattattgctgatgttgatgaacgcactagaaagaccggtgaggcttttgctgctggtttggctccagattgtgctattactgttcatcatcaagctgatacttcttccccagatccattgtttaacccattgaagactggtgtttgtcaattggatgttgctaacgttactagagctattttggaaagagctggtggttctattgctgattttactggtcattaccaaaccgcctttcgtgaattggaaagagttttgaactttccacaatccaacttgtgtttgaagagagaaaagcaagatgagtcctgttccttgacccaagctcttccatctgaattgaaggtttctgctgataacgtttctttgactggtgctgtttctttggcttctatgttgactgaaattttcttgttgcagcaggctcaaggtatgccagaaccaggttggggtagaattactgattctcatcaatggaacactttgttgtctttgcataacgctcaatttgacttgttggagagaactccagaagttgctagatctagagctactccattgttggatttgattaagactgctttgactccacatccaccacaaaagcaggcttacggtgttactttgccaacttctgttttgtttattgccggtcatgataccaacttggctaacttgggtggtgctttggaattgaactggactttgccaggtcaaccagataacactccaccaggtggtgaattggtttttgaaagatggagaagattgtccgataactctcaatggattcaagtttctttggtctttcagaccttgcagcaaatgagagataagactccattgtctttgaacactccaccaggtgaagttaagttgactttggctggttgtgaagaaagaaacgctcaaggtatgtgttctttggctggttttactcaaattgtcaacgaggctagaatcccagcttgttctttg

SEQ ID NO: 15 - protein, 410 aa, Artificial Sequence
  Phytase mutant
QSEPELKLESVVIVSRHGVRAPTKATQLMQDVTPDAWPTWPVKLGELTPRGGELIAYLGHYWRQRLVADELLPKKGCPQSGQVAIIADVDERTRKTGEAFAAGLAPDCAITVHHQADTSSPDPLFNPLKTGVCQLDVANVTRAILERAGGSIADFTGHYQTAFRELERVLNFPQSNLCLKREKQDESCSLTQALPSELKVSADNVSLTGAVSLASMLTEIFLLQQAQGMPEPGWGRITDSHQWNTLLSLHNAQFDLLQRTPEVARPRATPLLDLIKTALTPHPPQKQAYGVTLPTSVLFIAGHDTNLANLGGALELNWTLPGQPDNTPPGGELVFERWRRLSDNSQWIQVSLVFQTLQQMRDKTPLSLNTPPGEVKLTLAGCEERNAQGMCSLAGFTQIVNEARIPACSL

SEQ ID NO: 16 - DNA, 1230 bp, Artificial Sequence
  Nucleotide sequence encoding phytase mutant
caatctgaaccagaattgaagttggaatctgttgttattgtttcccgtcacggtgttagagccccaactaaggctactcaattgatgcaagatgttactccagatgcttggccaacttggccagttaagttgggtgaattgactccaagaggtggtgaattgattgcttacttgggtcattactggagacaaagattggttgctgatgaattgttgccaaagaagggttgtccacaatctggtcaagttgctattattgctgatgttgatgaacgcactagaaagaccggtgaggcttttgctgctggtttggctccagattgtgctattactgttcatcatcaagctgatacttcttccccagatccattgtttaacccattgaagactggtgtttgtcaattggatgttgctaacgttactagagctattttggaaagagctggtggttctattgctgattttactggtcattaccaaaccgcctttcgtgaattggaaagagttttgaactttccacaatccaacttgtgtttgaagagagaaaagcaagatgagtcctgttccttgacccaagctcttccatctgaattgaaggtttctgctgataacgtttctttgactggtgctgtttctttggcttctatgttgactgaaattttcttgttgcagcaggctcaaggtatgccagaaccaggttggggtagaattactgattctcatcaatggaacactttgttgtctttgcataacgctcaatttgacttgttgcaaagaactccagaagttgctagaccaagagctactccattgttggatttgattaagactgctttgactccacatccaccacaaaagcaggcttacggtgttactttgccaacttctgttttgtttattgccggtcatgataccaacttggctaacttgggtggtgctttggaattgaactggactttgccaggtcaaccagataacactccaccaggtggtgaattggtttttgaaagatggagaagattgtccgataactctcaatggattcaagtttctttggtctttcagaccttgcagcaaatgagagataagactccattgtctttgaacactccaccaggtgaagttaagttgactttggctggttgtgaagaaagaaacgctcaaggtatgtgttctttggctggttttactcaaattgtcaacgaggctagaatcccagcttgttctttg

SEQ ID NO: 17 - protein, 410 aa, Artificial Sequence
  Phytase mutant
QSEPELKLESVVIVSRHGVRAPTKATQLMQDVTPDPWPTWPVKLGELTPRGGELIAYLGHYWRQRLVADELLPKKGCPQSGQVAIIADVDERTRKTGEAFAAGLAPDCAITVHHQADTSSPDPLFNPLKTGVCQLDVANVTRAILERAGGSIADFTGHYQTAFRELERVLNFPQSNLCLKREKQDESCSLTQALPSELKVSADNVSLTGAWSLASMLTEIFLLQQAQGMPEPGWGRITDSHQWNTLLSLHNAQFDLLQRTPEVARSRATPLLDLIKTALTPHPPQKQAYGVTLPTSVLFIAGHDTNLANLGGALELNWTLPGQPDNTPPGGELVFERWRRLSDNSQWIQVSLVFQTLQQMRDKTPLSLNTPPGEVKLTLAGCEERNAQGMCSLAGFTQIVNEARIPACSL

SEQ ID NO: 18 - DNA, 1230 bp, Artificial Sequence
  Nucleotide sequence encoding phytase mutant
caatctgaaccagaattgaagttggaatctgttgttattgtttcccgtcacggtgttagagccccaactaaggctactcaattgatgcaagatgttactccagatccatggccaacttggccagttaagttgggtgaattgactccaagaggtggtgaattgattgcttacttgggtcattactggagacaaagattggttgctgatgaattgttgccaaagaagggttgtccacaatctggtcaagttgctattattgctgatgttgatgaacgcactagaaagaccggtgaggcttttgctgctggtttggctccagattgtgctattactgttcatcatcaagctgatacttcttccccagatccattgtttaacccattgaagactggtgtttgtcaattggatgttgctaacgttactagagctattttggaaagagctggtggttctattgctgattttactggtcattaccaaaccgcctttcgtgaattggaaagagttttgaactttccacaatccaacttgtgtttgaagagagaaaagcaagatgagtcctgttccttgacccaagctcttccatctgaattgaaggtttctgctgataacgtttctttgactggtgcttggtctttggcttctatgttgactgaaattttcttgttgcagcaggctcaaggtatgccagaaccaggttggggtagaattactgattctcatcaatggaacactttgttgtctttgcataacgctcaatttgacttgttgcaaagaactccagaagttgctagatctagagctactccattgttggatttgattaagactgctttgactccacatccaccacaaaagcaggcttacggtgttactttgccaacttctgttttgtttattgccggtcatgataccaacttggctaacttgggtggtgctttggaattgaactggactttgccaggtcaaccagataacactccaccaggtggtgaattggtttttgaaagatggagaagattgtccgataactctcaatggattcaagtttctttggtctttcagaccttgcagcaaatgagagataagactccattgtctttgaacactccaccaggtgaagttaagttgactttggctggttgtgaagaaagaaacgctcaaggtatgtgttctttggctggttttactcaaattgtcaacgaggctagaatcccagcttgttctttg

SEQ ID NO: 19 - protein, 410 aa, Artificial Sequence
  Phytase mutant
QSEPELKLESVVIVSRHGVRAPTKATQLMQDVTPDPWPTWPVKLGELTPRGGELIAYLGHYWRQRLVADELLPKKGCPQSGQVAIIADVDERTRKTGEAFAAGLAPDCAITVHHQADTSSPDPLFNPLKTGVCQLDVANVTRAILERAGGSIADFTGHYQTAFRELERVLNFPQSNLCLKREKQDESCSLTQALPSELKVSADNVSLTGAVSLASMLTEIFLLQQAQGMPEPGWGRITDSHQWNTLLSLHNAYFDLLQRTPEVARSRATPLLDLIKTALTPHPPQKQAYGVTLPTSVLFIAGHDTNLANLGGALELNWTLPGQPDNTPPGGELVFERWRRLSDNSQWIQVSLVFQTLQQMRDKTPLSLNTPPGEVKLTLAGCEERNAQGMCSLAGFTQIVNEARIPACSL

SEQ ID NO: 20 - DNA, 1230 bp, Artificial Sequence
  Nucleotide sequence encoding phytase mutant
caatctgaaccagaattgaagttggaatctgttgttattgtttcccgtcacggtgttagagccccaactaaggctactcaattgatgcaagatgttactccagatccatggccaacttggccagttaagttgggtgaattgactccaagaggtggtgaattgattgcttacttgggtcattactggagacaaagattggttgctgatgaattgttgccaaagaagggttgtccacaatctggtcaagttgctattattgctgatgttgatgaacgcactagaaagaccggtgaggcttttgctgctggtttggctccagattgtgctattactgttcatcatcaagctgatacttcttccccagatccattgtttaacccattgaagactggtgtttgtcaattggatgttgctaacgttactagagctattttggaaagagctggtggttctattgctgattttactggtcattaccaaaccgcctttcgtgaattggaaagagttttgaactttccacaatccaacttgtgtttgaagagagaaaagcaagatgagtcctgttccttgacccaagctcttccatctgaattgaaggtttctgctgataacgtttctttgactggtgctgtttctttggcttctatgttgactgaaattttcttgttgcagcaggctcaaggtatgccagaaccaggttggggtagaattactgattctcatcaatggaacactttgttgtctttgcataacgcttactttgacttgttgcaaagaactccagaagttgctagatctagagctactccattgttggatttgattaagactgctttgactccacatccaccacaaaagcaggcttacggtgttactttgccaacttctgttttgtttattgccggtcatgataccaacttggctaacttgggtggtgctttggaattgaactggactttgccaggtcaaccagataacactccaccaggtggtgaattggtttttgaaagatggagaagattgtccgataactctcaatggattcaagtttctttggtctttcagaccttgcagcaaatgagagataagactccattgtctttgaacactccaccaggtgaagttaagttgactttggctggttgtgaagaaagaaacgctcaaggtatgtgttctttggctggttttactcaaattgtcaacgaggctagaatcccagcttgttctttg

SEQ ID NO: 21 - protein, 410 aa, Artificial Sequence
  Phytase mutant
QSEPELKLESVVIVSRHGVRAPTKATQLMQDVTPDAWPTWPVKLGELTPRGGELIAYLGHYWRQRLVADELLPKKGCPQSGQVAIIADVDERTRKTGEAFAAGLAPDCAITVHHQADTSSPDPLFNPLKTGVCQLDVANVTRAILERAGGSIADFTGHYQTAFRELERVLNFPQSNLCLKREKQDESCSLTQALPSELKVSADNVSLTGAWSLASMLTEIFLLQQAQGMPEPGWGRITDSHQWNTLLSLHNAYFDLLQRTPEVARSRATPLLDLIKTALTPHPPQKQAYGVTLPTSVLFIAGHDTNLANLGGALELNWTLPGQPDNTPPGGELVFERWRRLSDNSQWIQVSLVFQTLQQMRDKTPLSLNTPPGEVKLTLAGCEERNAQGMCSLAGFTQIVNEARIPACSL

SEQ ID NO: 22 - DNA, 1230 bp, Artificial Sequence
  Nucleotide sequence encoding phytase mutant
caatctgaaccagaattgaagttggaatctgttgttattgtttcccgtcacggtgttagagccccaactaaggctactcaattgatgcaagatgttactccagatgcttggccaacttggccagttaagttgggtgaattgactccaagaggtggtgaattgattgcttacttgggtcattactggagacaaagattggttgctgatgaattgttgccaaagaagggttgtccacaatctggtcaagttgctattattgctgatgttgatgaacgcactagaaagaccggtgaggcttttgctgctggtttggctccagattgtgctattactgttcatcatcaagctgatacttcttccccagatccattgtttaacccattgaagactggtgtttgtcaattggatgttgctaacgttactagagctattttggaaagagctggtggttctattgctgattttactggtcattaccaaaccgcctttcgtgaattggaaagagttttgaactttccacaatccaacttgtgtttgaagagagaaaagcaagatgagtcctgttccttgacccaagctcttccatctgaattgaaggtttctgctgataacgtttctttgactggtgcttggtctttggcttctatgttgactgaaattttcttgttgcagcaggctcaaggtatgccagaaccaggttggggtagaattactgattctcatcaatggaacactttgttgtctttgcataacgcttactttgacttgttgcaaagaactccagaagttgctagatctagagctactccattgttggatttgattaagactgctttgactccacatccaccacaaaagcaggcttacggtgttactttgccaacttctgttttgtttattgccggtcatgataccaacttggctaacttgggtggtgctttggaattgaactggactttgccaggtcaaccagataacactccaccaggtggtgaattggtttttgaaagatggagaagattgtccgataactctcaatggattcaagtttctttggtctttcagaccttgcagcaaatgagagataagactccattgtctttgaacactccaccaggtgaagttaagttgactttggctggttgtgaagaaagaaacgctcaaggtatgtgttctttggctggttttactcaaattgtcaacgaggctagaatcccagcttgttctttg

SEQ ID NO: 23 - protein, 410 aa, Artificial Sequence
  Phytase mutant
QSEPELKLESVVIVSRHGVRAPTKATQLMQDVTPDPWPTWPVKLGELTPRGGELIAYLGHYWRQRLVADELLPKKGCPQSGQVAIIADVDERTRKTGEAFAAGLAPDCAITVHHQADTSSPDPLFNPLKTGVCQLDVANVTRAILERAGGSIADFTGHYQTAFRELERVLNFPQSNLCLKREKQDESCSLTQALPSELKVSADNVSLTGAWSLASMLTEIFLLQQAQGMPEPGWGRITDSHQWNTLLSLHNAYFDLLQRTPEVARSRATPLLDLIKTALTPHPPQKQAYGVTLPTSVLFIAGHDTNLANLGGALELNWTLPGQPDNTPPGGELVFERWRRLSDNSQWIQVSLVFQTLQQMRDKTPLSLNTPPGEVKLTLAGCEERNAQGMCSLAGFTQIVNEARIPACSL

SEQ ID NO: 24 - DNA, 1230 bp, Artificial Sequence
  Nucleotide sequence encoding phytase mutant
caatctgaaccagaattgaagttggaatctgttgttattgtttcccgtcacggtgttagagccccaactaaggctactcaattgatgcaagatgttactccagatccatggccaacttggccagttaagttgggtgaattgactccaagaggtggtgaattgattgcttacttgggtcattactggagacaaagattggttgctgatgaattgttgccaaagaagggttgtccacaatctggtcaagttgctattattgctgatgttgatgaacgcactagaaagaccggtgaggcttttgctgctggtttggctccagattgtgctattactgttcatcatcaagctgatacttcttccccagatccattgtttaacccattgaagactggtgtttgtcaattggatgttgctaacgttactagagctattttggaaagagctggtggttctattgctgattttactggtcattaccaaaccgcctttcgtgaattggaaagagttttgaactttccacaatccaacttgtgtttgaagagagaaaagcaagatgagtcctgttccttgacccaagctcttccatctgaattgaaggtttctgctgataacgtttctttgactggtgcttggtctttggcttctatgttgactgaaattttcttgttgcagcaggctcaaggtatgccagaaccaggttggggtagaattactgattctcatcaatggaacactttgttgtctttgcataacgcttactttgacttgttgcaaagaactccagaagttgctagatctagagctactccattgttggatttgattaagactgctttgactccacatccaccacaaaagcaggcttacggtgttactttgccaacttctgttttgtttattgccggtcatgataccaacttggctaacttgggtggtgctttggaattgaactggactttgccaggtcaaccagataacactccaccaggtggtgaattggtttttgaaagatggagaagattgtccgataactctcaatggattcaagtttctttggtctttcagaccttgcagcaaatgagagataagactccattgtctttgaacactccaccaggtgaagttaagttgactttggctggttgtgaagaaagaaacgctcaaggtatgtgttctttggctggttttactcaaattgtcaacgaggctagaatcccagcttgttctttg

SEQ ID NO: 25 - protein, 410 aa, Artificial Sequence
  Phytase mutant
QSEPELKLESVVIVSRHGVRAPTKATQLMQDVTPDPWPTWPVKLGELTPRGGELIAYLGHYWRQRLVADELLPKKGCPQSGQVAIIADVDERTRKTGEAFAAGLAPDCAITVHHQADTSSPDPLFEPLKTGVCQLDVANVTRAILERAGGSIADFTGHYQTAFRELERVLNFPQSNLCLKREKQDESCSLTQALPSELKVSADNVSLTGAWSLASMLTEIFLLQQAQGMPEPGWGRITDSHQWNTLLSLHNAYFDLLQRTPEVARSRATPLLDLIKTALTPHPPQKQAYGVTLPTSVLFIAGHDTNLANLGGALELNWTLPGQPDNTPPGGELVFERWRRLSDNSQWIQVSLVFQTLQQMRDKTPLSLNTPPGEVKLTLAGCEERNAQGMCSLAGFTQIVNEARIPACSL

SEQ ID NO: 26 - DNA, 1230 bp, Artificial Sequence
  Nucleotide sequence encoding phytase mutant
caatctgaaccagaattgaagttggaatctgttgttattgtttcccgtcacggtgttagagccccaactaaggctactcaattgatgcaagatgttactccagatccatggccaacttggccagttaagttgggtgaattgactccaagaggtggtgaattgattgcttacttgggtcattactggagacaaagattggttgctgatgaattgttgccaaagaagggttgtccacaatctggtcaagttgctattattgctgatgttgatgaacgcactagaaagaccggtgaggcttttgctgctggtttggctccagattgtgctattactgttcatcatcaagctgatacttcttccccagatccattgtttgagccattgaagactggtgtttgtcaattggatgttgctaacgttactagagctattttggaaagagctggtggttctattgctgattttactggtcattaccaaaccgcctttcgtgaattggaaagagttttgaactttccacaatccaacttgtgtttgaagagagaaaagcaagatgagtcctgttccttgacccaagctcttccatctgaattgaaggtttctgctgataacgtttctttgactggtgcttggtctttggcttctatgttgactgaaattttcttgttgcagcaggctcaaggtatgccagaaccaggttggggtagaattactgattctcatcaatggaacactttgttgtctttgcataacgcttactttgacttgttgcaaagaactccagaagttgctagatctagagctactccattgttggatttgattaagactgctttgactccacatccaccacaaaagcaggcttacggtgttactttgccaacttctgttttgtttattgccggtcatgataccaacttggctaacttgggtggtgctttggaattgaactggactttgccaggtcaaccagataacactccaccaggtggtgaattggtttttgaaagatggagaagattgtccgataactctcaatggattcaagtttctttggtctttcagaccttgcagcaaatgagagataagactccattgtctttgaacactccaccaggtgaagttaagttgactttggctggttgtgaagaaagaaacgctcaaggtatgtgttctttggctggttttactcaaattgtcaacgaggctagaatcccagcttgttctttg

SEQ ID NO: 27 - DNA, 32 bp, Artificial Sequence
  M0-F1 primer
ggcgaattccagtcagaaccagagttgaagtt

SEQ ID NO: 28 - DNA, 32 bp, Artificial Sequence
  M0-R1 primer
atagcggccgcttacaaggaacaagcagggat